European Patent Application EP 4 810 522 A1, published September 23, 2026. Title: 融合蛋白及其用途. Applicant: 维康平生（北京）生物科技有限公司. The sequence listing filed with the application follows.

SEQUENCE LISTING (23 sequences)

SEQ ID NO: 1 - protein, 28 aa, synthetic construct
MELTIFILRLAIYILTFPLYLLNFLGLW

SEQ ID NO: 2 - protein, 27 aa, synthetic construct
MDALVLFLQLLVLLLTLPLHLLALLGC

SEQ ID NO: 3 - protein, 28 aa, synthetic construct
MGAQLSTLGHMVLFPVWFLYSLLMKLFQ

SEQ ID NO: 4 - protein, 42 aa, synthetic construct
MQIPVLTRILPAQLLLWSRVRLWRLMMWLWPLQKILLQLVSH

SEQ ID NO: 5 - protein, 28 aa, synthetic construct
MNIILEILLLLITIIYSYLESLVKFFIP

SEQ ID NO: 6 - protein, 40 aa, synthetic construct
MLTIGQRVKNLASLIVQGVSNKAHDHVIDPINERARNYLE

SEQ ID NO: 7 - protein, 65 aa, synthetic construct
MPEELAELREKFTADELRKVAEAYLKVASDLYTSLAERGEDTVERIRKQPVVEEGIGRAETAFGD

SEQ ID NO: 8 - protein, 51 aa, synthetic construct
MQDILESVVVTLHAICLLIISTIRNCFPMGWLLRKDVRGQTVLITGSGSGL

SEQ ID NO: 9 - protein, 38 aa, synthetic construct
MKFLLDILLLLPLLIVCSLESFVKLFIPKRRKSVTGEI

SEQ ID NO: 10 - protein, 21 aa, synthetic construct
MGIFSRFADIVNANINALLEK

SEQ ID NO: 11 - protein, 22 aa, synthetic construct
MNLFERFSRVVKSYANALISSF

SEQ ID NO: 12 - protein, 49 aa, synthetic construct
MWSSLFGWTSSNAKNKESPTKAIVRLREHINLLSKKQSHLRTQITNQEN

SEQ ID NO: 13 - protein, 30 aa, synthetic construct
MAVNFLRMSARVDAVAARVQTAVTMGKVTK

SEQ ID NO: 14 - protein, 20 aa, synthetic construct
MRRLLRILRLLRRIIRRRLR

SEQ ID NO: 15 - protein, 20 aa, synthetic construct
MRFLRRILRLLRRIIRRVLR

SEQ ID NO: 16 - protein, 20 aa, synthetic construct
MEFLESVLSGLVRIIRRVLE

SEQ ID NO: 17 - protein, 5 aa, synthetic construct
CRGDK

SEQ ID NO: 18 - protein, 12 aa, synthetic construct
THRPPMWSPVWP

SEQ ID NO: 19 - protein, 11 aa, synthetic construct
HLRKLRKRLLR

SEQ ID NO: 20 - protein, 12 aa, synthetic construct
FCDGFYACYKDV

SEQ ID NO: 21 - protein, 10 aa, synthetic construct
LGASWHRPDK

SEQ ID NO: 22 - protein, 13 aa, synthetic construct
CTVALPGGYVRVC

SEQ ID NO: 23 - protein, 8 aa, synthetic construct
FCDWKTCT